European Patent Application EP 4 190 806 A1, published June 7, 2023. Title: Heterodimeric Fc fusion proteins, and related compositions, uses and methods. Applicant: Medytox Inc. The sequence listing filed with the application follows.

SEQUENCE LISTING (15 sequences)

SEQ ID NO: 1 - protein, 217 aa, Homo sapiens
APELLGGPSVFLFPPKPKDTLMISRTPEVTCVVVDVSHEDPEVKFNWYVDGVEVHNAKTKPREEQYNSTYRVVSVLTVLHQDWLNGKEYKCKVSNKALPAPIEKTISKAKGQPREPQVYTLPPSREEMTKNQVSLTCLVKGFYPSDIAVEWESNGQPENNYKTTPPVLDSDGSFFLYSKLTVDKSRWQQGNVFSCSVMHEALHNHYTQKSLSLSPGK

SEQ ID NO: 2 - protein, 217 aa, Artificial Sequence
  Human IgG1 Fc(Knob; S354C, T366W)
APELLGGPSVFLFPPKPKDTLMISRTPEVTCVVVDVSHEDPEVKFNWYVDGVEVHNAKTKPREEQYNSTYRVVSVLTVLHQDWLNGKEYKCKVSNKALPAPIEKTISKAKGQPREPQVYTLPPCREEMTKNQVSLWCLVKGFYPSDIAVEWESNGQPENNYKTTPPVLDSDGSFFLYSKLTVDKSRWQQGNVFSCSVMHEALHNHYTQKSLSLSPGK

SEQ ID NO: 3 - protein, 217 aa, Artificial Sequence
  Human IgG1 Fc(Hole; Y349C, T366S, L368A, Y407V)
APELLGGPSVFLFPPKPKDTLMISRTPEVTCVVVDVSHEDPEVKFNWYVDGVEVHNAKTKPREEQYNSTYRVVSVLTVLHQDWLNGKEYKCKVSNKALPAPIEKTISKAKGQPREPQVCTLPPSREEMTKNQVSLSCAVKGFYPSDIAVEWESNGQPENNYKTTPPVLDSDGSFFLVSKLTVDKSRWQQGNVFSCSVMHEALHNHYTQKSLSLSPGK

SEQ ID NO: 4 - protein, 562 aa, Artificial Sequence
  IL-1R-hinge region-CH2-CH3(S354C, T366W)
MKVLLRLICFIALLISSLEADKCKEREEKIILVSSANEIDVRPCPLNPNEHKGTITWYKDDSKTPVSTEQASRIHQHKEKLWFVPAKVEDSGHYYCVVRNSSYCLRIKISAKFVENEPNLCYNAQAIFKQKLPVAGDGGLVCPYMEFFKNENNELPKLQWYKDCKPLLLDNIHFSGVKDRLIVMNVAEKHRGNYTCHASYTYLGKQYPITRVIEFITLEENKPTRPVIVSPANETMEVDLGSQIQLICNVTGQLSDIAYWKWNGSVIDEDDPVLGEDYYSVENPANKRRSTLITVLNISEIESRFYKHPFTCFAKNTHGIDAAYIQLIYPVTNSGDKTHTCPPCPAPELLGGPSVFLFPPKPKDTLMISRTPEVTCVVVDVSHEDPEVKFNWYVDGVEVHNAKTKPREEQYNSTYRVVSVLTVLHQDWLNGKEYKCKVSNKALPAPIEKTISKAKGQPREPQVYTLPPCREEMTKNQVSLWCLVKGFYPSDIAVEWESNGQPENNYKTTPPVLDSDGSFFLYSKLTVDKSRWQQGNVFSCSVMHEALHNHYTQKSLSLSPGK

SEQ ID NO: 5 - protein, 697 aa, Artificial Sequence
  IL-1RAcP-hinge region-CH2-CH3(Y349C, T366S, L368A, Y407V)
MTLLWCVVSLYFYGILQSDASERCDDWGLDTMRQIQVFEDEPARIKCPLFEHFLKFNYSTAHSAGLTLIWYWTRQDRDLEEPINFRLPENRISKEKDVLWFRPTLLNDTGNYTCMLRNTTYCSKVAFPLEVVQKDSCFNSPMKLPVHKLYIEYGIQRITCPNVDGYFPSSVKPTITWYMGCYKIQNFNNVIPEGMNLSFLIALISNNGNYTCVVTYPENGRTFHLTRTLTVKVVGSPKNAVPPVIHSPNDHVVYEKEPGEELLIPCTVYFSFLMDSRNEVWWTIDGKKPDDITIDVTINESISHSRTEDETRTQILSIKKVTSEDLKRSYVCHARSAKGEVAKAAKVKQKVPAPRYTVEQPKAAPGQPKAAPSVTLFPPSSEELQANKATLVCLISDFYPGAVTVAWKADSSPVKAGVETTTPSKQSNNKYAASSYLSLTPEQWKSHRSYSCQVTHEGSTVEKTVAPTESDKTHTCPPCPAPELLGGPSVFLFPPKPKDTLMISRTPEVTCVVVDVSHEDPEVKFNWYVDGVEVHNAKTKPREEQYNSTYRVVSVLTVLHQDWLNGKEYKCKVSNKALPAPIEKTISKAKGQPREPQVCTLPPSREEMTKNQVSLSCAVKGFYPSDIAVEWESNGQPENNYKTTPPVLDSDGSFFLVSKLTVDKSRWQQGNVFSCSVMHEALHNHYTQKSLSLSPGK

SEQ ID NO: 6 - protein, 107 aa, Homo sapiens
RTVAAPSVFIFPPSDEQLKSGTASVVCLLNNFYPREAKVQWKVDNALQSGNSQESVTEQDSKDSTYSLSSTLTLSKADYEKHKVYACEVTHQGLSSPVTKSFNRGES

SEQ ID NO: 7 - protein, 104 aa, Homo sapiens
QPKAAPSVTLFPPSSEELQANKATLVCLISDFYPGAVTVAWKADSSPVKAGVETTTPSKQSNNKYAASSYLSLTPEQWKSHRSYSCQVTHEGSTVEKTVAPTES

SEQ ID NO: 8 - protein, 674 aa, Artificial Sequence
  IL-1R-kappa constant region-hinge region-CH2-CH3 (S354C, T366W)
MKVLLRLICFIALLISSLEADKCKEREEKIILVSSANEIDVRPCPLNPNEHKGTITWYKDDSKTPVSTEQASRIHQHKEKLWFVPAKVEDSGHYYCVVRNSSYCLRIKISAKFVENEPNLCYNAQAIFKQKLPVAGDGGLVCPYMEFFKNENNELPKLQWYKDCKPLLLDNIHFSGVKDRLIVMNVAEKHRGNYTCHASYTYLGKQYPITRVIEFITLEENKPTRPVIVSPANETMEVDLGSQIQLICNVTGQLSDIAYWKWNGSVIDEDDPVLGEDYYSVENPANKRRSTLITVLNISEIESRFYKHPFTCFAKNTHGIDAAYIQLIYPVTNSGTVAAPRTVAAPSVFIFPPSDEQLKSGTASVVCLLNNFYPREAKVQWKVDNALQSGNSQESVTEQDSKDSTYSLSSTLTLSKADYEKHKVYACEVTHQGLSSPVTKSFNRGESDKTHTCPPCPAPELLGGPSVFLFPPKPKDTLMISRTPEVTCVVVDVSHEDPEVKFNWYVDGVEVHNAKTKPREEQYNSTYRVVSVLTVLHQDWLNGKEYKCKVSNKALPAPIEKTISKAKGQPREPQVYTLPPCREEMTKNQVSLWCLVKGFYPSDIAVEWESNGQPENNYKTTPPVLDSDGSFFLYSKLTVDKSRWQQGNVFSCSVMHEALHNHYTQKSLSLSPGK

SEQ ID NO: 9 - protein, 697 aa, Artificial Sequence; identical to SEQ ID NO: 5
  IL-1RAcP-lambda constant region-hinge region-CH2-CH3 (Y349C, T366S, L368A, Y407V)

SEQ ID NO: 10 - protein, 735 aa, Artificial Sequence
  IL1R-hinge region-CH2-CH3(S354C, T366W, K447del)-(G4S)2-IL18BP
MKVLLRLICFIALLISSLEADKCKEREEKIILVSSANEIDVRPCPLNPNEHKGTITWYKDDSKTPVSTEQASRIHQHKEKLWFVPAKVEDSGHYYCVVRNSSYCLRIKISAKFVENEPNLCYNAQAIFKQKLPVAGDGGLVCPYMEFFKNENNELPKLQWYKDCKPLLLDNIHFSGVKDRLIVMNVAEKHRGNYTCHASYTYLGKQYPITRVIEFITLEENKPTRPVIVSPANETMEVDLGSQIQLICNVTGQLSDIAYWKWNGSVIDEDDPVLGEDYYSVENPANKRRSTLITVLNISEIESRFYKHPFTCFAKNTHGIDAAYIQLIYPVTNSGDKTHTCPPCPAPELLGGPSVFLFPPKPKDTLMISRTPEVTCVVVDVSHEDPEVKFNWYVDGVEVHNAKTKPREEQYNSTYRVVSVLTVLHQDWLNGKEYKCKVSNKALPAPIEKTISKAKGQPREPQVYTLPPCREEMTKNQVSLWCLVKGFYPSDIAVEWESNGQPENNYKTTPPVLDSDGSFFLYSKLTVDKSRWQQGNVFSCSVMHEALHNHYTQKSLSLSPGGGGGSGGGGSTPVSQTTTAATASVRSTKDPCPSQPPVFPAAKQCPALEVTWPEVEVPLNGTLSLSCVACSRFPNFSILYWLGNGSFIEHLPGRLWEGSTSRERGSTGTQLCKALVLEQLTPALHSTNFSCVLVDPEQVVQRHVVLAQLWAGLRATLPPTQEALPSSHSSPQQQG

SEQ ID NO: 11 - protein, 759 aa, Artificial Sequence
  IL1RAcP-hinge region-CH2-CH3(Y349C, T366S, L368A, Y407V, K447del)-(G4S)2-IL18BP
MTLLWCVVSLYFYGILQSDASERCDDWGLDTMRQIQVFEDEPARIKCPLFEHFLKFNYSTAHSAGLTLIWYWTRQDRDLEEPINFRLPENRISKEKDVLWFRPTLLNDTGNYTCMLRNTTYCSKVAFPLEVVQKDSCFNSPMKLPVHKLYIEYGIQRITCPNVDGYFPSSVKPTITWYMGCYKIQNFNNVIPEGMNLSFLIALISNNGNYTCVVTYPENGRTFHLTRTLTVKVVGSPKNAVPPVIHSPNDHVVYEKEPGEELLIPCTVYFSFLMDSRNEVWWTIDGKKPDDITIDVTINESISHSRTEDETRTQILSIKKVTSEDLKRSYVCHARSAKGEVAKAAKVKQKVPAPRYTVEDKTHTCPPCPAPELLGGPSVFLFPPKPKDTLMISRTPEVTCVVVDVSHEDPEVKFNWYVDGVEVHNAKTKPREEQYNSTYRVVSVLTVLHQDWLNGKEYKCKVSNKALPAPIEKTISKAKGQPREPQVCTLPPSREEMTKNQVSLSCAVKGFYPSDIAVEWESNGQPENNYKTTPPVLDSDGSFFLVSKLTVDKSRWQQGNVFSCSVMHEALHNHYTQKSLSLSPGGGGGSGGGGSTPVSQTTTAATASVRSTKDPCPSQPPVFPAAKQCPALEVTWPEVEVPLNGTLSLSCVACSRFPNFSILYWLGNGSFIEHLPGRLWEGSTSRERGSTGTQLCKALVLEQLTPALHSTNFSCVLVDPEQVVQRHVVLAQLWAGLRATLPPTQEALPSSHSSPQQQG

SEQ ID NO: 12 - protein, 847 aa, Artificial Sequence
  IL1R-kappa constant region-hinge region-CH2-CH3(S354C, T366W, K447del)-(G4S)2-IL18BP
MKVLLRLICFIALLISSLEADKCKEREEKIILVSSANEIDVRPCPLNPNEHKGTITWYKDDSKTPVSTEQASRIHQHKEKLWFVPAKVEDSGHYYCVVRNSSYCLRIKISAKFVENEPNLCYNAQAIFKQKLPVAGDGGLVCPYMEFFKNENNELPKLQWYKDCKPLLLDNIHFSGVKDRLIVMNVAEKHRGNYTCHASYTYLGKQYPITRVIEFITLEENKPTRPVIVSPANETMEVDLGSQIQLICNVTGQLSDIAYWKWNGSVIDEDDPVLGEDYYSVENPANKRRSTLITVLNISEIESRFYKHPFTCFAKNTHGIDAAYIQLIYPVTNSGTVAAPRTVAAPSVFIFPPSDEQLKSGTASVVCLLNNFYPREAKVQWKVDNALQSGNSQESVTEQDSKDSTYSLSSTLTLSKADYEKHKVYACEVTHQGLSSPVTKSFNRGESDKTHTCPPCPAPELLGGPSVFLFPPKPKDTLMISRTPEVTCVVVDVSHEDPEVKFNWYVDGVEVHNAKTKPREEQYNSTYRVVSVLTVLHQDWLNGKEYKCKVSNKALPAPIEKTISKAKGQPREPQVYTLPPCREEMTKNQVSLWCLVKGFYPSDIAVEWESNGQPENNYKTTPPVLDSDGSFFLYSKLTVDKSRWQQGNVFSCSVMHEALHNHYTQKSLSLSPGGGGGSGGGGSTPVSQTTTAATASVRSTKDPCPSQPPVFPAAKQCPALEVTWPEVEVPLNGTLSLSCVACSRFPNFSILYWLGNGSFIEHLPGRLWEGSTSRERGSTGTQLCKALVLEQLTPALHSTNFSCVLVDPEQVVQRHVVLAQLWAGLRATLPPTQEALPSSHSSPQQQG

SEQ ID NO: 13 - protein, 735 aa, Artificial Sequence; identical to SEQ ID NO: 10
  IL1RAcP-lambda constant region-hinge region-CH2-CH3(Y349C, T366S, L368A, Y407V, K447del)-(G4S)2-IL18BP

SEQ ID NO: 14 - protein, 831 aa, Artificial Sequence
  IL1R-kappa constant region-hinge region-CH2-CH3(S354C, T366W, K447A)-(G4S)4G-TGFbetaRII
MKVLLRLICFIALLISSLEADKCKEREEKIILVSSANEIDVRPCPLNPNEHKGTITWYKDDSKTPVSTEQASRIHQHKEKLWFVPAKVEDSGHYYCVVRNSSYCLRIKISAKFVENEPNLCYNAQAIFKQKLPVAGDGGLVCPYMEFFKNENNELPKLQWYKDCKPLLLDNIHFSGVKDRLIVMNVAEKHRGNYTCHASYTYLGKQYPITRVIEFITLEENKPTRPVIVSPANETMEVDLGSQIQLICNVTGQLSDIAYWKWNGSVIDEDDPVLGEDYYSVENPANKRRSTLITVLNISEIESRFYKHPFTCFAKNTHGIDAAYIQLIYPVTNSGTVAAPRTVAAPSVFIFPPSDEQLKSGTASVVCLLNNFYPREAKVQWKVDNALQSGNSQESVTEQDSKDSTYSLSSTLTLSKADYEKHKVYACEVTHQGLSSPVTKSFNRGESDKTHTCPPCPAPELLGGPSVFLFPPKPKDTLMISRTPEVTCVVVDVSHEDPEVKFNWYVDGVEVHNAKTKPREEQYNSTYRVVSVLTVLHQDWLNGKEYKCKVSNKALPAPIEKTISKAKGQPREPQVYTLPPCREEMTKNQVSLWCLVKGFYPSDIAVEWESNGQPENNYKTTPPVLDSDGSFFLYSKLTVDKSRWQQGNVFSCSVMHEALHNHYTQKSLSLSPGAGGGGSGGGGSGGGGSGGGGSGIPPHVQKSVNNDMIVTDNNGAVKFPQLCKFCDVRFSTCDNQKSCMSNCSITSICEKPQEVCVAVWRKNDENITLETVCHDPKLPYHDFILEDAASPKCIMKEKKKPGETFFMCSCSSDECNDNIIFSEEYNTSNPD

SEQ ID NO: 15 - protein, 853 aa, Artificial Sequence
  IL1RAcP-lambda constant region-hinge region-CH2-CH3(Y349C, T366S, L368A, Y407V, K447A)-(G4S)4G-TGFbetaRII
MTRLTVLALLAGLLASSRASERCDDWGLDTMRQIQVFEDEPARIKCPLFEHFLKFNYSTAHSAGLTLIWYWTRQDRDLEEPINFRLPENRISKEKDVLWFRPTLLNDTGNYTCMLRNTTYCSKVAFPLEVVQKDSCFNSPMKLPVHKLYIEYGIQRITCPNVDGYFPSSVKPTITWYMGCYKIQNFNNVIPEGMNLSFLIALISNNGNYTCVVTYPENGRTFHLTRTLTVKVVGSPKNAVPPVIHSPNDHVVYEKEPGEELLIPCTVYFSFLMDSRNEVWWTIDGKKPDDITIDVTINESISHSRTEDETRTQILSIKKVTSEDLKRSYVCHARSAKGEVAKAAKVKQKVPAPRYTVEQPKAAPGQPKAAPSVTLFPPSSEELQANKATLVCLISDFYPGAVTVAWKADSSPVKAGVETTTPSKQSNNKYAASSYLSLTPEQWKSHRSYSCQVTHEGSTVEKTVAPTESDKTHTCPPCPAPELLGGPSVFLFPPKPKDTLMISRTPEVTCVVVDVSHEDPEVKFNWYVDGVEVHNAKTKPREEQYNSTYRVVSVLTVLHQDWLNGKEYKCKVSNKALPAPIEKTISKAKGQPREPQVCTLPPSREEMTKNQVSLSCAVKGFYPSDIAVEWESNGQPENNYKTTPPVLDSDGSFFLVSKLTVDKSRWQQGNVFSCSVMHEALHNHYTQKSLSLSPGAGGGGSGGGGSGGGGSGGGGSGIPPHVQKSVNNDMIVTDNNGAVKFPQLCKFCDVRFSTCDNQKSCMSNCSITSICEKPQEVCVAVWRKNDENITLETVCHDPKLPYHDFILEDAASPKCIMKEKKKPGETFFMCSCSSDECNDNIIFSEEYNTSNPD